European Patent Specification EP 3 828 204 B1, published October 22, 2025. Title: FUSION PROTEINS OF HUMAN PROTEIN FRAGMENTS TO CREATE ORDERLY MULTIMERIZED IMMUNOGLOBULIN FC COMPOSITIONS WITH ENHANCED COMPLEMENT BINDING. Applicant: Gliknik Inc. Application EP. The sequence listing filed with the application follows.

SEQUENCE LISTING (87 sequences)

SEQ ID NO: 1 - protein, 20 aa, Artificial Sequence
  Leader Sequence
METDTLLLWVLLLWVPGSTG

SEQ ID NO: 2 - protein, 232 aa, Homo sapiens
EPKSCDKTHTCPPCPAPELLGGPSVFLFPPKPKDTLMISRTPEVTCVVVDVSHEDPEVKFNWYVDGVEVHNAKTKPREEQYNSTYRVVSVLTVLHQDWLNGKEYKCKVSNKALPAPIEKTISKAKGQPREPQVYTLPPSREEMTKNQVSLTCLVKGFYPSDIAVEWESNGQPENNYKTTPPVLDSDGSFFLYSKLTVDKSRWQQGNVFSCSVMHEALHNHYTQKSLSLSPGK

SEQ ID NO: 3 - protein, 232 aa, Homo sapiens
EPKSCDKTHTCPPCPAPELLGGPSVFLFPPKPKDTLMISRTPEVTCVVVDVSHEDPEVKFNWYVDGVEVHNAKTKPREEQYNSTYRVVSVLTVLHQDWLNGKEYKCKVSNKALPAPIEKTISKAKGQPREPQVYTLPPSRDELTKNQVSLTCLVKGFYPSDIAVEWESNGQPENNYKTTPPVLDSDGSFFLYSKLTVDKSRWQQGNVFSCSVMHEALHNHYTQKSLSLSPGK

SEQ ID NO: 4 - protein, 12 aa, Homo sapiens
ERKCCVECPPCP

SEQ ID NO: 5 - protein, 41 aa, Homo sapiens
GGGSIKQIEDKIEEILSKIYHIENEIARIKKLIGERGHGGG

SEQ ID NO: 6 - protein, 16 aa, Artificial Sequence
  GPP multimerization domain
GPPGPPGPPGPPGPPG

SEQ ID NO: 7 - protein, 264 aa, Homo sapiens
METDTLLLWVLLLWVPGSTGEPKSCDKTHTCPPCPAPELLGGPSVFLFPPKPKDTLMISRTPEVTCVVVDVSHEDPEVKFNWYVDGVEVHNAKTKPREEQYNSTYRVVSVLTVLHQDWLNGKEYKCKVSNKALPAPIEKTISKAKGQPREPQVYTLPPSREEMTKNQVSLTCLVKGFYPSDIAVEWESNGQPENNYKTTPPVLDSDGSFFLYSKLTVDKSRWQQGNVFSCSVMHEALHNHYTQKSLSLSPGKERKCCVECPPCP

SEQ ID NO: 8 - protein, 264 aa, Homo sapiens
METDTLLLWVLLLWVPGSTGEPKSCDKTHTCPPCPAPELLGGPSVFLFPPKPKDTLMISRTPEVTCVVVDVSHEDPEVKFNWYVDGVEVHNAKTKPREEQYNSTYRVVSVLTVLHQDWLNGKEYKCKVSNKALPAPIEKTISKAKGQPREPQVYTLPPSRDELTKNQVSLTCLVKGFYPSDIAVEWESNGQPENNYKTTPPVLDSDGSFFLYSKLTVDKSRWQQGNVFSCSVMHEALHNHYTQKSLSLSPGKERKCCVECPPCP

SEQ ID NO: 9 - protein, 263 aa, Homo sapiens
METDTLLLWVLLLVPGSTGERKCCVECPPCPEPKSCDKTHTCPPCPAPELLGGPSVFLFPPKPKDTLMISRTPEVTCVVVDVSHEDPEVKFNWYVDGVEVHNAKTKPREEQYNSTYRVVSVLTVLHQDWLNGKEYKCKVSNKALPAPIEKTISKAKGQPREPQVYTLPPSREEMTKNQVSLTCLVKGFYPSDIAVEWESNGQPENNYKTTPPVLDSDGSFFLYSKLTVDKSRWQQGNVFSCSVMHEALHNHYTQKSLSLSPGK

SEQ ID NO: 10 - protein, 264 aa, Homo sapiens
METDTLLLWVLLLWVPGSTGEPKSCDKTHTCPPCPAPPLLRGPSVFLFPPKPKDTLMISRTPEVTCVVVDVEFEDPEVKFNWYVDGVEVHNAKTKPREEQYNSTYRVVSVLTVLHQDWLNGKEYKCKVTNKALPAPIEKTISKAKGQPREPQVYTLPPSRDELTKNQVSLTCLVKGFYPSDIAVEWESNGQPENNYKTTPPVLDSDGSFFLYSKLTVDKSRWQQGNVFSCSVMHEALHNHYTQKSLSLSPGKERKCCVECPPCP

SEQ ID NO: 11 - protein, 264 aa, Homo sapiens
METDTLLLWVLLLWVPGSTGEPKSCDKTHTCPPCPAPPLLRGPSVFLFPPKPKDTLMISRTPEVTCVVVDVEFEDPEVKFNWYVDGVEVHNAKTKPREEQYNSTYRVVSVLTVLHQDWLNGKEYKCKVTNKALPAPIEKTISKAKGQPREPQVYTLPPSREEMTKNQVSLTCLVKGFYPSDIAVEWESNGQPENNYKTTPPVLDSDGSFFLYSKLTVDKSRWQQGNVFSCSVMHEALHNHYTQKSLSLSPGKERKCCVECPPCP

SEQ ID NO: 12 - protein, 264 aa, Homo sapiens
METDTLLLWVLLLWVPGSTGEPKSCDKTHTCPPCPAPELLRGPSVFLFPPKPKDTLMISRTPEVTCVVVDVEFEDPEVKFNWYVDGVEVHNAKTKPREEQYNSTYRVVSVLTVLHQDWLNGKEYKCKVTNKALPAPIEKTISKAKGQPREPQVYTLPPSRDELTKNQVSLTCLVKGFYPSDIAVEWESNGQPENNYKTTPPVLDSDGSFFLYSKLTVDKSRWQQGNVFSCSVMHEALHNHYTQKSLSLSPGKERKCCVECPPCP

SEQ ID NO: 13 - protein, 264 aa, Homo sapiens
METDTLLLWVLLLWVPGSTGEPKSCDKTHTCPPCPAPELLGGPSVFLFPPKPKDTLMISRTPEVTCVVVDVEFEDPEVKFNWYVDGVEVHNAKTKPREEQYNSTYRVVSVLTVLHQDWLNGKEYKCKVTNKALPAPIEKTISKAKGQPREPQVYTLPPSRDELTKNQVSLTCLVKGFYPSDIAVEWESNGQPENNYKTTPPVLDSDGSFFLYSKLTVDKSRWQQGNVFSCSVMHEALHNHYTQKSLSLSPGKERKCCVECPPCP

SEQ ID NO: 14 - protein, 264 aa, Homo sapiens
METDTLLLWVLLLWVPGSTGEPKSCDKTHTCPPCPAPELLGGPSVFLFPPKPKDTLMISRTPEVTCVVVDVEFEDPEVKFNWYVDGVEVHNAKTKPREEQYASTYRVVSVLTVLHQDWLNGKEYKCKVTNKALPAPIEKTISKAKGQPREPQVYTLPPSRDELTKNQVSLTCLVKGFYPSDIAVEWESNGQPENNYKTTPPVLDSDGSFFLYSKLTVDKSRWQQGNVFSCSVMHEALHNHYTQKSLSLSPGKERKCCVECPPCP

SEQ ID NO: 15 - protein, 264 aa, Homo sapiens
METDTLLLWVLLLWVPGSTGEPKSCDKTHTCPPCPAPELLGGPSVFLFPPKPKDTLMISRTPEVTCVVVDVEFEDPEVKFNWYVDGVEVHNAKTKPREEQYASTYRVVSVLTVLHQDWLNGKEYKCKVTNKALPAPIEKTISKAKGQPREPQVYTLPPSREEMTKNQVSLTCLVKGFYPSDIAVEWESNGQPENNYKTTPPVLDSDGSFFLYSKLTVDKSRWQQGNVFSCSVMHEALHNHYTQKSLSLSPGKERKCCVECPPCP

SEQ ID NO: 16 - protein, 264 aa, Homo sapiens
METDTLLLWVLLLWVPGSTGEPKSCDKTHTCPPCPAPPLLRGPSVFLFPPKPKDTLMISRTPEVTCVVVDVSHEDPEVKFNWYVDGVEVHNAKTKPREEQYNSTYRVVSVLTVLHQDWLNGKEYKCKVSNKALPAPIEKTISKAKGQPREPQVYTLPPSRDELTKNQVSLTCLVKGFYPSDIAVEWESNGQPENNYKTTPPVLDSDGSFFLYSKLTVDKSRWQQGNVFSCSVMHEALHNHYTQKSLSLSPGKERKCCVECPPCP

SEQ ID NO: 17 - protein, 264 aa, Homo sapiens
METDTLLLWVLLLWVPGSTGERKCCVECPPCPEPKSCDKTHTCPPCPAPELLGGPSVFLFPPKPKDTLMISRTPEVTCVVVDVEFEDPEVKFNWYVDGVEVHNAKTKPREEQYNSTYRVVSVLTVLHQDWLNGKEYKCKVTNKALPAPIEKTISKAKGQPREPQVYTLPPSREEMTKNQVSLTCLVKGFYPSDIAVEWESNGQPENNYKTTPPVLDSDGSFFLYSKLTVDKSRWQQGNVFSCSVMHEALHNHYTQKSLSLSPGK

SEQ ID NO: 18 - protein, 264 aa, Homo sapiens
METDTLLLWVLLLWVPGSTGEPKSCDKTHTCPPCPAPELLGGPSVFLFPPKPKDTLMISRTPEVTCVVVAVEFEDPEVKFNWYVDGVEVHNAKTKPREEQYNSTYRVVSVLTVLHQDWLNGKEYKCKVTNKALPAPIEKTISKAKGQPREPQVYTLPPSRDELTKNQVSLTCLVKGFYPSDIAVEWESNGQPENNYKTTPPVLDSDGSFFLYSKLTVDKSRWQQGNVFSCSVMHEALHNHYTQKSLSLSPGKERKCCVECPPCP

SEQ ID NO: 19 - protein, 264 aa, Homo sapiens
METDTLLLWVLLLWVPGSTGEPKSCDKTHTCPPCPAPPVAGGPSVFLFPPKPKDTLMISRTPEVTCVVVDVEFEDPEVKFNWYVDGVEVHNAKTKPREEQYASTYRVVSVLTVLHQDWLNGKEYKCKVTNKALPAPIEKTISKAKGQPREPQVYTLPPSRDELTKNQVSLTCLVKGFYPSDIAVEWESNGQPENNYKTTPPVLDSDGSFFLYSKLTVDKSRWQQGNVFSCSVMHEALHNHYTQKSLSLSPGKERKCCVECPPCP

SEQ ID NO: 20 - protein, 264 aa, Homo sapiens
METDTLLLWVLLLWVPGSTGEPKSCDKTHTCPPCPAPELLGGDSVFLFPPKPKDTLMISRTPEVTCVVVDVEFEDPEVKFNWYVDGVEVHNAKTKPREEQYASTYRVVSVLTVLHQDWLNGKEYKCKVTNKALPAPIEKTISKAKGQPREPQVYTLPPSRDELTKNQVSLTCLVKGFYPSDIAVEWESNGQPENNYKTTPPVLDSDGSFFLYSKLTVDKSRWQQGNVFSCSVMHEALHNHYTQKSLSLSPGKERKCCVECPPCP

SEQ ID NO: 21 - protein, 264 aa, Homo sapiens
METDTLLLWVLLLWVPGSTGEPKSCDKTHTCPPCPAPEAAGGPSVFLFPPKPKDTLMISRTPEVTCVVVDVEFEDPEVKFNWYVDGVEVHNAKTKPREEQYASTYRVVSVLTVLHQDWLNGKEYKCKVTNKALPAPIEKTISKAKGQPREPQVYTLPPSRDELTKNQVSLTCLVKGFYPSDIAVEWESNGQPENNYKTTPPVLDSDGSFFLYSKLTVDKSRWQQGNVFSCSVMHEALHNHYTQKSLSLSPGKERKCCVECPPCP

SEQ ID NO: 22 - protein, 264 aa, Homo sapiens
METDTLLLWVLLLWVPGSTGEPKSCDKTHTCPPCPAPEAAGGPSVFLFPPKPKDTLMISRTPEVTCVVVDVEFEDPEVKFNWYVDGVEVHNAKTKPREEQYASTYRVVSVLTVLHQDWLNGKEYKCKVTNKALPAPIEKTISKAKGQPREPQVYTLPPSREEMTKNQVSLTCLVKGFYPSDIAVEWESNGQPENNYKTTPPVLDSDGSFFLYSKLTVDKSRWQQGNVFSCSVMHEALHNHYTQKSLSLSPGKERKCCVECPPCP

SEQ ID NO: 23 - protein, 264 aa, Homo sapiens
METDTLLLWVLLLWVPGSTGEPKSCDKTHTCPPCPAPPLLRGPSVFLFPPKPKDTLMISRTPEVTCVVVDVEFEDPEVKFNWYVDGVEVHNAKTKPREEQYNSTYRVVSVLTVLHQDWLNGKEYKCKVTNKAFPAPIEKTISKAKGQPREPQVYTLPPSRDELTKNQVSLTCLVKGFYPSDIAVEWESNGQPENNYKTTPPVLDSDGSFFLYSKLTVDKSRWQQGNVFSCSVMHEALHNHYTQKSLSLSPGKERKCCVECPPCP

SEQ ID NO: 24 - protein, 264 aa, Homo sapiens
METDTLLLWVLLLWVPGSTGEPKSCDKTHTCPPCPAPELLGGDSVFLFPPKPKDTLMISRTPEVTCVVVGVEFEDPEVKFNWYVDGVEVHNAKTKPREEQYNSTYRVVSVLTVLHQDWLNGKEYKCKVTNKALPAPIEKTISKAKGQPREPQVYTLPPSREEMTKNQVSLTCLVKGFYPSDIAVEWESNGQPENNYKTTPPVLDSDGSFFLYSKLTVDKSRWQQGNVFSCSVMHEALHNHYTQKSLSLSPGKERKCCVECPPCP

SEQ ID NO: 25 - protein, 264 aa, Homo sapiens
METDTLLLWVLLLWVPGSTGEPKSCDKTHTCPPCPAPELLGGDSVFLFPPKPKDTLMISRTPEVTCVVVWVEFEDPEVKFNWYVDGVEVHNAKTKPREEQYNSTYRVVSVLTVLHQDWLNGKEYKCKVTNKALPAPIEKTISKAKGQPREPQVYTLPPSREEMTKNQVSLTCLVKGFYPSDIAVEWESNGQPENNYKTTPPVLDSDGSFFLYSKLTVDKSRWQQGNVFSCSVMHEALHNHYTQKSLSLSPGKERKCCVECPPCP

SEQ ID NO: 26 - protein, 263 aa, Homo sapiens
METDTLLLWVLLLWVPGSTGEPKSCDKTHTCPPCPAPPVAGPSVFLFPPKPKDTLMISRTPEVTCVVVDVEFEDPEVKFNWYVDGVEVHNAKTKPREEQYASTYRVVSVLTVLHQDWLNGKEYKCKVTNKAFPAPIEKTISKAKGQPREPQVYTLPPSRDELTKNQVSLTCLVKGFYPSDIAVEWESNGQPENNYKTTPPVLDSDGSFFLYSKLTVDKSRWQQGNVFSCSVMHEALHNHYTQKSLSLSPGKERKCCVECPPCP

SEQ ID NO: 27 - protein, 264 aa, Homo sapiens
METDTLLLWVLLLWVPGSTGEPKSCDKTHTCPPCPAPELLGGDSVFLFPPKPKDTLMISRTPEVTCVVVDVEFEDPEVKFNWYVDGVEVHNAKTKPREEQYNSTYRVVSVLTVLHQDWLNGKEYKCKVTNKALPAPIEKTISKAKGQPREPQVYTLPPSRDELTKNQVSLTCLVKGFYPSDIAVEWESNGQPENNYKTTPPVLDSDGSFFLYSKLTVDKSRWQQGNVFSCSVMHEALHNHYTQKSLSLSPGKERKCCVECPPCP

SEQ ID NO: 28 - protein, 264 aa, Homo sapiens
METDTLLLWVLLLWVPGSTGEPKSCDKTHTCPPCPAPPLLQGPSVFLFPPKPKDTLMISRTPEVTCVVVDVSFEDPEVKFNWYVDGVEVHNAKTKPREEQYNSTYRVVSVLTVLHQDWLNGKEYKCKVTNKALPAPIEKTISKAKGQPREPQVYTLPPSRDELTKNQVSLTCLVKGFYPSDIAVEWESNGQPENNYKTTPPVLDSDGSFFLYSKLTVDKSRWQQGNVFSCSVMHEALHNHYTQKSLSLSPGKERKCCVECPPCP

SEQ ID NO: 29 - protein, 264 aa, Homo sapiens
METDTLLLWVLLLWVPGSTGEPKSCDKTHTCPPCPAPPLLRGPSVFLFPPKPKDTLMISRTPEVTCVVVDVSFEDPEVKFNWYVDGVEVHNAKTKPREEQYNSTYRVVSVLTVLHQDWLNGKEYKCKVTNKALPAPIEKTISKAKGQPREPQVYTLPPSRDELTKNQVSLTCLVKGFYPSDIAVEWESNGQPENNYKTTPPVLDSDGSFFLYSKLTVDKSRWQQGNVFSCSVMHEALHNHYTQKSLSLSPGKERKCCVECPPCP

SEQ ID NO: 30 - protein, 264 aa, Homo sapiens
METDTLLLWVLLLWVPGSTGEPKSCDKTHTCPPCPAPPLLHGPSVFLFPPKPKDTLMISRTPEVTCVVVDVSFEDPEVKFNWYVDGVEVHNAKTKPREEQYNSTYRVVSVLTVLHQDWLNGKEYKCKVTNKALPAPIEKTISKAKGQPREPQVYTLPPSRDELTKNQVSLTCLVKGFYPSDIAVEWESNGQPENNYKTTPPVLDSDGSFFLYSKLTVDKSRWQQGNVFSCSVMHEALHNHYTQKSLSLSPGKERKCCVECPPCP

SEQ ID NO: 31 - protein, 264 aa, Homo sapiens
METDTLLLWVLLLWVPGSTGEPKSCDKTHTCPPCPAPPLLNGPSVFLFPPKPKDTLMISRTPEVTCVVVDVSFEDPEVKFNWYVDGVEVHNAKTKPREEQYNSTYRVVSVLTVLHQDWLNGKEYKCKVTNKALPAPIEKTISKAKGQPREPQVYTLPPSRDELTKNQVSLTCLVKGFYPSDIAVEWESNGQPENNYKTTPPVLDSDGSFFLYSKLTVDKSRWQQGNVFSCSVMHEALHNHYTQKSLSLSPGKERKCCVECPPCP

SEQ ID NO: 32 - protein, 264 aa, Homo sapiens
METDTLLLWVLLLWVPGSTGEPKSCDKTHTCPPCPAPPLLKGPSVFLFPPKPKDTLMISRTPEVTCVVVDVSFEDPEVKFNWYVDGVEVHNAKTKPREEQYNSTYRVVSVLTVLHQDWLNGKEYKCKVTNKALPAPIEKTISKAKGQPREPQVYTLPPSRDELTKNQVSLTCLVKGFYPSDIAVEWESNGQPENNYKTTPPVLDSDGSFFLYSKLTVDKSRWQQGNVFSCSVMHEALHNHYTQKSLSLSPGKERKCCVECPPCP

SEQ ID NO: 33 - protein, 264 aa, Homo sapiens
METDTLLLWVLLLWVPGSTGEPKSCDKTHTCPPCPAPPLLGGPSVFLFPPKPKDTLMISRTPEVTCVVVDVRFEDPEVKFNWYVDGVEVHNAKTKPREEQYNSTYRVVSVLTVLHQDWLNGKEYKCKVTNKALPAPIEKTISKAKGQPREPQVYTLPPSRDELTKNQVSLTCLVKGFYPSDIAVEWESNGQPENNYKTTPPVLDSDGSFFLYSKLTVDKSRWQQGNVFSCSVMHEALHNHYTQKSLSLSPGKERKCCVECPPCP

SEQ ID NO: 34 - protein, 264 aa, Homo sapiens
METDTLLLWVLLLWVPGSTGEPKSCDKTHTCPPCPAPPLLGGPSVFLFPPKPKDTLMISRTPEVTCVVVDVNFEDPEVKFNWYVDGVEVHNAKTKPREEQYNSTYRVVSVLTVLHQDWLNGKEYKCKVTNKALPAPIEKTISKAKGQPREPQVYTLPPSRDELTKNQVSLTCLVKGFYPSDIAVEWESNGQPENNYKTTPPVLDSDGSFFLYSKLTVDKSRWQQGNVFSCSVMHEALHNHYTQKSLSLSPGKERKCCVECPPCP

SEQ ID NO: 35 - protein, 264 aa, Homo sapiens
METDTLLLWVLLLWVPGSTGEPKSCDKTHTCPPCPAPPLLGGPSVFLFPPKPKDTLMISRTPEVTCVVVDVKFEDPEVKFNWYVDGVEVHNAKTKPREEQYNSTYRVVSVLTVLHQDWLNGKEYKCKVTNKALPAPIEKTISKAKGQPREPQVYTLPPSRDELTKNQVSLTCLVKGFYPSDIAVEWESNGQPENNYKTTPPVLDSDGSFFLYSKLTVDKSRWQQGNVFSCSVMHEALHNHYTQKSLSLSPGKERKCCVECPPCP

SEQ ID NO: 36 - protein, 264 aa, Homo sapiens
METDTLLLWVLLLWVPGSTGEPKSCDKTHTCPPCPAPPLLDGPSVFLFPPKPKDTLMISRTPEVTCVVVDVRFEDPEVKFNWYVDGVEVHNAKTKPREEQYNSTYRVVSVLTVLHQDWLNGKEYKCKVTNKALPAPIEKTISKAKGQPREPQVYTLPPSRDELTKNQVSLTCLVKGFYPSDIAVEWESNGQPENNYKTTPPVLDSDGSFFLYSKLTVDKSRWQQGNVFSCSVMHEALHNHYTQKSLSLSPGKERKCCVECPPCP

SEQ ID NO: 37 - protein, 264 aa, Homo sapiens
METDTLLLWVLLLWVPGSTGEPKSCDKTHTCPPCPAPPLLRGPSVFLFPPKPKDTLMISRTPEVTCVVVDVRFEDPEVKFNWYVDGVEVHNAKTKPREEQYNSTYRVVSVLTVLHQDWLNGKEYKCKVTNKALPAPIEKTISKAKGQPREPQVYTLPPSRDELTKNQVSLTCLVKGFYPSDIAVEWESNGQPENNYKTTPPVLDSDGSFFLYSKLTVDKSRWQQGNVFSCSVMHEALHNHYTQKSLSLSPGKERKCCVECPPCP

SEQ ID NO: 38 - protein, 264 aa, Homo sapiens
METDTLLLWVLLLWVPGSTGEPKSCDKTHTCPPCPAPPLLRGPSVFLFPPKPKDTLMISRTPEVTCVVVDVDFEDPEVKFNWYVDGVEVHNAKTKPREEQYNSTYRVVSVLTVLHQDWLNGKEYKCKVTNKALPAPIEKTISKAKGQPREPQVYTLPPSRDELTKNQVSLTCLVKGFYPSDIAVEWESNGQPENNYKTTPPVLDSDGSFFLYSKLTVDKSRWQQGNVFSCSVMHEALHNHYTQKSLSLSPGKERKCCVECPPCP

SEQ ID NO: 39 - protein, 264 aa, Homo sapiens
METDTLLLWVLLLWVPGSTGEPKSCDKTHTCPPCPAPPLLEGPSVFLFPPKPKDTLMISRTPEVTCVVVDVRFEDPEVKFNWYVDGVEVHNAKTKPREEQYNSTYRVVSVLTVLHQDWLNGKEYKCKVTNKALPAPIEKTISKAKGQPREPQVYTLPPSRDELTKNQVSLTCLVKGFYPSDIAVEWESNGQPENNYKTTPPVLDSDGSFFLYSKLTVDKSRWQQGNVFSCSVMHEALHNHYTQKSLSLSPGKERKCCVECPPCP

SEQ ID NO: 40 - protein, 264 aa, Homo sapiens
METDTLLLWVLLLWVPGSTGEPKSCDKTHTCPPCPAPPLLHGPSVFLFPPKPKDTLMISRTPEVTCVVVDVKFEDPEVKFNWYVDGVEVHNAKTKPREEQYNSTYRVVSVLTVLHQDWLNGKEYKCKVTNKALPAPIEKTISKAKGQPREPQVYTLPPSRDELTKNQVSLTCLVKGFYPSDIAVEWESNGQPENNYKTTPPVLDSDGSFFLYSKLTVDKSRWQQGNVFSCSVMHEALHNHYTQKSLSLSPGKERKCCVECPPCP

SEQ ID NO: 41 - protein, 264 aa, Homo sapiens
METDTLLLWVLLLWVPGSTGEPKSCDKTHTCPPCPAPPLLQGPSVFLFPPKPKDTLMISRTPEVTCVVVDVQFEDPEVKFNWYVDGVEVHNAKTKPREEQYNSTYRVVSVLTVLHQDWLNGKEYKCKVTNKALPAPIEKTISKAKGQPREPQVYTLPPSRDELTKNQVSLTCLVKGFYPSDIAVEWESNGQPENNYKTTPPVLDSDGSFFLYSKLTVDKSRWQQGNVFSCSVMHEALHNHYTQKSLSLSPGKERKCCVECPPCP

SEQ ID NO: 42 - protein, 264 aa, Homo sapiens
METDTLLLWVLLLWVPGSTGEPKSCDKTHTCPPCPAPPLLRGPSVFLFPPKPKDTLMISRTPEVTCVVVDVKFEDPEVKFNWYVDGVEVHNAKTKPREEQYNSTYRVVSVLTVLHQDWLNGKEYKCKVTNKALPAPIEKTISKAKGQPREPQVYTLPPSRDELTKNQVSLTCLVKGFYPSDIAVEWESNGQPENNYKTTPPVLDSDGSFFLYSKLTVDKSRWQQGNVFSCSVMHEALHNHYTQKSLSLSPGKERKCCVECPPCP

SEQ ID NO: 43 - protein, 264 aa, Homo sapiens
METDTLLLWVLLLWVPGSTGEPKSCDKTHTCPPCPAPPLLRGPSVFLFPPKPKDTLMISRTPEVTCVVVDVQFEDPEVKFNWYVDGVEVHNAKTKPREEQYNSTYRVVSVLTVLHQDWLNGKEYKCKVTNKALPAPIEKTISKAKGQPREPQVYTLPPSRDELTKNQVSLTCLVKGFYPSDIAVEWESNGQPENNYKTTPPVLDSDGSFFLYSKLTVDKSRWQQGNVFSCSVMHEALHNHYTQKSLSLSPGKERKCCVECPPCP

SEQ ID NO: 44 - protein, 264 aa, Homo sapiens
METDTLLLWVLLLWVPGSTGEPKSCDKTHTCPPCPAPPLLDGPSVFLFPPKPKDTLMISRTPEVTCVVVDVKFEDPEVKFNWYVDGVEVHNAKTKPREEQYNSTYRVVSVLTVLHQDWLNGKEYKCKVTNKALPAPIEKTISKAKGQPREPQVYTLPPSRDELTKNQVSLTCLVKGFYPSDIAVEWESNGQPENNYKTTPPVLDSDGSFFLYSKLTVDKSRWQQGNVFSCSVMHEALHNHYTQKSLSLSPGKERKCCVECPPCP

SEQ ID NO: 45 - protein, 264 aa, Homo sapiens
METDTLLLWVLLLWVPGSTGEPKSCDKTHTCPPCPAPPLLHGPSVFLFPPKPKDTLMISRTPEVTCVVVDVQFEDPEVKFNWYVDGVEVHNAKTKPREEQYNSTYRVVSVLTVLHQDWLNGKEYKCKVTNKALPAPIEKTISKAKGQPREPQVYTLPPSRDELTKNQVSLTCLVKGFYPSDIAVEWESNGQPENNYKTTPPVLDSDGSFFLYSKLTVDKSRWQQGNVFSCSVMHEALHNHYTQKSLSLSPGKERKCCVECPPCP

SEQ ID NO: 46 - protein, 264 aa, Homo sapiens
METDTLLLWVLLLWVPGSTGEPKSCDKTHTCPPCPAPPLLQGPSVFLFPPKPKDTLMISRTPEVTCVVVDVRFEDPEVKFNWYVDGVEVHNAKTKPREEQYNSTYRVVSVLTVLHQDWLNGKEYKCKVTNKALPAPIEKTISKAKGQPREPQVYTLPPSRDELTKNQVSLTCLVKGFYPSDIAVEWESNGQPENNYKTTPPVLDSDGSFFLYSKLTVDKSRWQQGNVFSCSVMHEALHNHYTQKSLSLSPGKERKCCVECPPCP

SEQ ID NO: 47 - protein, 264 aa, Homo sapiens
METDTLLLWVLLLWVPGSTGEPKSCDKTHTCPPCPAPPLLKGPSVFLFPPKPKDTLMISRTPEVTCVVVDVKFEDPEVKFNWYVDGVEVHNAKTKPREEQYNSTYRVVSVLTVLHQDWLNGKEYKCKVTNKALPAPIEKTISKAKGQPREPQVYTLPPSRDELTKNQVSLTCLVKGFYPSDIAVEWESNGQPENNYKTTPPVLDSDGSFFLYSKLTVDKSRWQQGNVFSCSVMHEALHNHYTQKSLSLSPGKERKCCVECPPCP

SEQ ID NO: 48 - protein, 264 aa, Homo sapiens
METDTLLLWVLLLWVPGSTGEPKSCDKTHTCPPCPAPPLLKGPSVFLFPPKPKDTLMISRTPEVTCVVVDVNFEDPEVKFNWYVDGVEVHNAKTKPREEQYNSTYRVVSVLTVLHQDWLNGKEYKCKVTNKALPAPIEKTISKAKGQPREPQVYTLPPSRDELTKNQVSLTCLVKGFYPSDIAVEWESNGQPENNYKTTPPVLDSDGSFFLYSKLTVDKSRWQQGNVFSCSVMHEALHNHYTQKSLSLSPGKERKCCVECPPCP

SEQ ID NO: 49 - protein, 264 aa, Homo sapiens
METDTLLLWVLLLWVPGSTGEPKSCDKTHTCPPCPAPPLLNGPSVFLFPPKPKDTLMISRTPEVTCVVVDVEFEDPEVKFNWYVDGVEVHNAKTKPREEQYNSTYRVVSVLTVLHQDWLNGKEYKCKVTNKALPAPIEKTISKAKGQPREPQVYTLPPSRDELTKNQVSLTCLVKGFYPSDIAVEWESNGQPENNYKTTPPVLDSDGSFFLYSKLTVDKSRWQQGNVFSCSVMHEALHNHYTQKSLSLSPGKERKCCVECPPCP

SEQ ID NO: 50 - protein, 264 aa, Homo sapiens
METDTLLLWVLLLWVPGSTGEPKSCDKTHTCPPCPAPPLLNGPSVFLFPPKPKDTLMISRTPEVTCVVVDVKFEDPEVKFNWYVDGVEVHNAKTKPREEQYNSTYRVVSVLTVLHQDWLNGKEYKCKVTNKALPAPIEKTISKAKGQPREPQVYTLPPSRDELTKNQVSLTCLVKGFYPSDIAVEWESNGQPENNYKTTPPVLDSDGSFFLYSKLTVDKSRWQQGNVFSCSVMHEALHNHYTQKSLSLSPGKERKCCVECPPCP

SEQ ID NO: 51 - protein, 264 aa, Homo sapiens
METDTLLLWVLLLWVPGSTGEPKSCDKTHTCPPCPAPPLLRGPSVFLFPPKPKDTLMISRTPEVTCVVVDVNFEDPEVKFNWYVDGVEVHNAKTKPREEQYNSTYRVVSVLTVLHQDWLNGKEYKCKVTNKALPAPIEKTISKAKGQPREPQVYTLPPSRDELTKNQVSLTCLVKGFYPSDIAVEWESNGQPENNYKTTPPVLDSDGSFFLYSKLTVDKSRWQQGNVFSCSVMHEALHNHYTQKSLSLSPGKERKCCVECPPCP

SEQ ID NO: 52 - protein, 264 aa, Homo sapiens
METDTLLLWVLLLWVPGSTGEPKSCDKTHTCPPCPAPELLGGPSVFLFPPKPKDTLMISRTPEVTCVVVDVSFEDPEVKFNWYVDGVEVHNAKTKPREEQYNSAYRVVSVLTVLHQDWLNGKEYKCKVTNKALPAPIEKTISKAKGQPREPQVYTLPPSRDELTKNQVSLTCLVKGFYPSDIAVEWESNGQPENNYKTTPPVLDSDGSFFLYSKLTVDKSRWQQGNVFSCSVMHEALHNHYTQKSLSLSPGKERKCCVECPPCP

SEQ ID NO: 53 - protein, 264 aa, Homo sapiens
METDTLLLWVLLLWVPGSTGEPKSCDKTHTCPPCPAPELLGGPSVFLFPPKPKDTLMISRTPEVTCVVVDVRFEDPEVKFNWYVDGVEVHNAKTKPREEQYNSAYRVVSVLTVLHQDWLNGKEYKCKVTNKALPAPIEKTISKAKGQPREPQVYTLPPSRDELTKNQVSLTCLVKGFYPSDIAVEWESNGQPENNYKTTPPVLDSDGSFFLYSKLTVDKSRWQQGNVFSCSVMHEALHNHYTQKSLSLSPGKERKCCVECPPCP

SEQ ID NO: 54 - protein, 264 aa, Homo sapiens
METDTLLLWVLLLWVPGSTGEPKSCDKTHTCPPCPAPELLGGPSVFLFPPKPKDTLMISRTPEVTCVVVDVKFEDPEVKFNWYVDGVEVHNAKTKPREEQYNSAYRVVSVLTVLHQDWLNGKEYKCKVTNKALPAPIEKTISKAKGQPREPQVYTLPPSRDELTKNQVSLTCLVKGFYPSDIAVEWESNGQPENNYKTTPPVLDSDGSFFLYSKLTVDKSRWQQGNVFSCSVMHEALHNHYTQKSLSLSPGKERKCCVECPPCP

SEQ ID NO: 55 - protein, 264 aa, Homo sapiens
METDTLLLWVLLLWVPGSTGEPKSCDKTHTCPPCPAPELLGGPSVFLFPPKPKDTLMISRTPEVTCVVVDVNFEDPEVKFNWYVDGVEVHNAKTKPREEQYNSAYRVVSVLTVLHQDWLNGKEYKCKVTNKALPAPIEKTISKAKGQPREPQVYTLPPSRDELTKNQVSLTCLVKGFYPSDIAVEWESNGQPENNYKTTPPVLDSDGSFFLYSKLTVDKSRWQQGNVFSCSVMHEALHNHYTQKSLSLSPGKERKCCVECPPCP

SEQ ID NO: 56 - protein, 264 aa, Homo sapiens
METDTLLLWVLLLWVPGSTGEPKSCDKTHTCPPCPAPELLGGPSVFLFPPKPKDTLMISRTPEVTCVVVDVSFEDPEVKFNWYVDGVEVHNAKTKPREEQYASTYRVVSVLTVLHQDWLNGKEYKCKVTNKALPAPIEKTISKAKGQPREPQVYTLPPSRDELTKNQVSLTCLVKGFYPSDIAVEWESNGQPENNYKTTPPVLDSDGSFFLYSKLTVDKSRWQQGNVFSCSVMHEALHNHYTQKSLSLSPGKERKCCVECPPCP

SEQ ID NO: 57 - protein, 264 aa, Homo sapiens
METDTLLLWVLLLWVPGSTGEPKSCDKTHTCPPCPAPELLGGPSVFLFPPKPKDTLMISRTPEVTCVVVDVKFEDPEVKFNWYVDGVEVHNAKTKPREEQYASTYRVVSVLTVLHQDWLNGKEYKCKVTNKALPAPIEKTISKAKGQPREPQVYTLPPSRDELTKNQVSLTCLVKGFYPSDIAVEWESNGQPENNYKTTPPVLDSDGSFFLYSKLTVDKSRWQQGNVFSCSVMHEALHNHYTQKSLSLSPGKERKCCVECPPCP

SEQ ID NO: 58 - protein, 264 aa, Homo sapiens
METDTLLLWVLLLWVPGSTGEPKSCDKTHTCPPCPAPELLGGPSVFLFPPKPKDTLMISRTPEVTCVVVDVRFEDPEVKFNWYVDGVEVHNAKTKPREEQYASTYRVVSVLTVLHQDWLNGKEYKCKVTNKALPAPIEKTISKAKGQPREPQVYTLPPSRDELTKNQVSLTCLVKGFYPSDIAVEWESNGQPENNYKTTPPVLDSDGSFFLYSKLTVDKSRWQQGNVFSCSVMHEALHNHYTQKSLSLSPGKERKCCVECPPCP

SEQ ID NO: 59 - protein, 264 aa, Homo sapiens
METDTLLLWVLLLWVPGSTGEPKSCDKTHTCPPCPAPELLGGPSVFLFPPKPKDTLMISRTPEVTCVVVDVDFEDPEVKFNWYVDGVEVHNAKTKPREEQYASTYRVVSVLTVLHQDWLNGKEYKCKVTNKALPAPIEKTISKAKGQPREPQVYTLPPSRDELTKNQVSLTCLVKGFYPSDIAVEWESNGQPENNYKTTPPVLDSDGSFFLYSKLTVDKSRWQQGNVFSCSVMHEALHNHYTQKSLSLSPGKERKCCVECPPCP

SEQ ID NO: 60 - protein, 264 aa, Homo sapiens
METDTLLLWVLLLWVPGSTGEPKSCDKTHTCPPCPAPELLGGPSVFLFPPKPKDTLMISRTPEVTCVVVDVQFEDPEVKFNWYVDGVEVHNAKTKPREEQYASTYRVVSVLTVLHQDWLNGKEYKCKVTNKALPAPIEKTISKAKGQPREPQVYTLPPSRDELTKNQVSLTCLVKGFYPSDIAVEWESNGQPENNYKTTPPVLDSDGSFFLYSKLTVDKSRWQQGNVFSCSVMHEALHNHYTQKSLSLSPGKERKCCVECPPCP

SEQ ID NO: 61 - protein, 264 aa, Homo sapiens
METDTLLLWVLLLWVPGSTGEPKSCDKTHTCPPCPAPELLRGPSVFLFPPKPKDTLMISRTPEVTCVVVDVSHEDPEVKFNWYVDGVEVHNAKTKPREEQYNSTYRVVSVLTVLHQDWLNGKEYKCKVSNKALPAPIEKTISKAKGQPREPQVYTLPPSRDELTKNQVSLTCLVKGFYPSDIAVEWESNGQPENNYKTTPPVLDSDGSFFLYSKLTVDKSRWQQGNVFSCSVMHEALHNHYTQKSLSLSPGKERKCCVECPPCP

SEQ ID NO: 62 - protein, 264 aa, Homo sapiens
METDTLLLWVLLLWVPGSTGEPKSCDKTHTCPPCPAPPVAGGPSVFLFPPKPKDTLMISRTPEVTCVVVDVEFEDPEVKFNWYVDGVEVHNAKTKPREEQYNSTYRVVSVLTVLHQDWLNGKEYKCKVTNKALPAPIEKTISKAKGQPREPQVYTLPPSRDELTKNQVSLTCLVKGFYPSDIAVEWESNGQPENNYKTTPPVLDSDGSFFLYSKLTVDKSRWQQGNVFSCSVMHEALHNHYTQKSLSLSPGKERKCCVECPPCP

SEQ ID NO: 63 - protein, 264 aa, Homo sapiens
METDTLLLWVLLLWVPGSTGEPKSCDKTHTCPPCPAPEAAGGPSVFLFPPKPKDTLMISRTPEVTCVVVDVEFEDPEVKFNWYVDGVEVHNAKTKPREEQYNSTYRVVSVLTVLHQDWLNGKEYKCKVTNKALPAPIEKTISKAKGQPREPQVYTLPPSRDELTKNQVSLTCLVKGFYPSDIAVEWESNGQPENNYKTTPPVLDSDGSFFLYSKLTVDKSRWQQGNVFSCSVMHEALHNHYTQKSLSLSPGKERKCCVECPPCP

SEQ ID NO: 64 - protein, 264 aa, Homo sapiens
METDTLLLWVLLLWVPGSTGERKCCVECPPCPEPKSCDKTHTCPPCPAPELLGGPSVFLFPPKPKDTLMISRTPEVTCVVVDVEFEDPEVKFNWYVDGVEVHNAKTKPREEQYNSTYRVVSVLTVLHQDWLNGKEYKCKVTNKAFPAPIEKTISKAKGQPREPQVYTLPPSRDELTKNQVSLTCLVKGFYPSDIAVEWESNGQPENNYKTTPPVLDSDGSFFLYSKLTVDKSRWQQGNVFSCSVMHEALHNHYTQKSLSLSPGK

SEQ ID NO: 65 - protein, 264 aa, Homo sapiens
METDTLLLWVLLLWVPGSTGEPKSCDKTHTCPPCPAPPLLEGPSVFLFPPKPKDTLMISRTPEVTCVVVDVSFEDPEVKFNWYVDGVEVHNAKTKPREEQYNSTYRVVSVLTVLHQDWLNGKEYKCKVTNKALPAPIEKTISKAKGQPREPQVYTLPPSRDELTKNQVSLTCLVKGFYPSDIAVEWESNGQPENNYKTTPPVLDSDGSFFLYSKLTVDKSRWQQGNVFSCSVMHEALHNHYTQKSLSLSPGKERKCCVECPPCP

SEQ ID NO: 66 - protein, 264 aa, Homo sapiens
METDTLLLWVLLLWVPGSTGEPKSCDKTHTCPPCPAPPLLDGPSVFLFPPKPKDTLMISRTPEVTCVVVDVSFEDPEVKFNWYVDGVEVHNAKTKPREEQYNSTYRVVSVLTVLHQDWLNGKEYKCKVTNKALPAPIEKTISKAKGQPREPQVYTLPPSRDELTKNQVSLTCLVKGFYPSDIAVEWESNGQPENNYKTTPPVLDSDGSFFLYSKLTVDKSRWQQGNVFSCSVMHEALHNHYTQKSLSLSPGKERKCCVECPPCP

SEQ ID NO: 67 - protein, 264 aa, Homo sapiens
METDTLLLWVLLLWVPGSTGEPKSCDKTHTCPPCPAPPLLGGPSVFLFPPKPKDTLMISRTPEVTCVVVDVQFEDPEVKFNWYVDGVEVHNAKTKPREEQYNSTYRVVSVLTVLHQDWLNGKEYKCKVTNKALPAPIEKTISKAKGQPREPQVYTLPPSRDELTKNQVSLTCLVKGFYPSDIAVEWESNGQPENNYKTTPPVLDSDGSFFLYSKLTVDKSRWQQGNVFSCSVMHEALHNHYTQKSLSLSPGKERKCCVECPPCP

SEQ ID NO: 68 - protein, 264 aa, Homo sapiens
METDTLLLWVLLLWVPGSTGEPKSCDKTHTCPPCPAPPLLGGPSVFLFPPKPKDTLMISRTPEVTCVVVDVDFEDPEVKFNWYVDGVEVHNAKTKPREEQYNSTYRVVSVLTVLHQDWLNGKEYKCKVTNKALPAPIEKTISKAKGQPREPQVYTLPPSRDELTKNQVSLTCLVKGFYPSDIAVEWESNGQPENNYKTTPPVLDSDGSFFLYSKLTVDKSRWQQGNVFSCSVMHEALHNHYTQKSLSLSPGKERKCCVECPPCP

SEQ ID NO: 69 - protein, 264 aa, Homo sapiens
METDTLLLWVLLLWVPGSTGEPKSCDKTHTCPPCPAPPLLGGPSVFLFPPKPKDTLMISRTPEVTCVVVDVHFEDPEVKFNWYVDGVEVHNAKTKPREEQYNSTYRVVSVLTVLHQDWLNGKEYKCKVTNKALPAPIEKTISKAKGQPREPQVYTLPPSRDELTKNQVSLTCLVKGFYPSDIAVEWESNGQPENNYKTTPPVLDSDGSFFLYSKLTVDKSRWQQGNVFSCSVMHEALHNHYTQKSLSLSPGKERKCCVECPPCP

SEQ ID NO: 70 - protein, 264 aa, Homo sapiens
METDTLLLWVLLLWVPGSTGEPKSCDKTHTCPPCPAPPLLGGPSVFLFPPKPKDTLMISRTPEVTCVVVDVEFEDPEVKFNWYVDGVEVHNAKTKPREEQYNSTYRVVSVLTVLHQDWLNGKEYKCKVTNKALPAPIEKTISKAKGQPREPQVYTLPPSRDELTKNQVSLTCLVKGFYPSDIAVEWESNGQPENNYKTTPPVLDSDGSFFLYSKLTVDKSRWQQGNVFSCSVMHEALHNHYTQKSLSLSPGKERKCCVECPPCP

SEQ ID NO: 71 - protein, 264 aa, Homo sapiens
METDTLLLWVLLLWVPGSTGEPKSCDKTHTCPPCPAPPLLDGPSVFLFPPKPKDTLMISRTPEVTCVVVDVQFEDPEVKFNWYVDGVEVHNAKTKPREEQYNSTYRVVSVLTVLHQDWLNGKEYKCKVTNKALPAPIEKTISKAKGQPREPQVYTLPPSRDELTKNQVSLTCLVKGFYPSDIAVEWESNGQPENNYKTTPPVLDSDGSFFLYSKLTVDKSRWQQGNVFSCSVMHEALHNHYTQKSLSLSPGKERKCCVECPPCP

SEQ ID NO: 72 - protein, 264 aa, Homo sapiens
METDTLLLWVLLLWVPGSTGEPKSCDKTHTCPPCPAPPLLQGPSVFLFPPKPKDTLMISRTPEVTCVVVDVDFEDPEVKFNWYVDGVEVHNAKTKPREEQYNSTYRVVSVLTVLHQDWLNGKEYKCKVTNKALPAPIEKTISKAKGQPREPQVYTLPPSRDELTKNQVSLTCLVKGFYPSDIAVEWESNGQPENNYKTTPPVLDSDGSFFLYSKLTVDKSRWQQGNVFSCSVMHEALHNHYTQKSLSLSPGKERKCCVECPPCP

SEQ ID NO: 73 - protein, 264 aa, Homo sapiens
METDTLLLWVLLLWVPGSTGEPKSCDKTHTCPPCPAPPLLDGPSVFLFPPKPKDTLMISRTPEVTCVVVDVDFEDPEVKFNWYVDGVEVHNAKTKPREEQYNSTYRVVSVLTVLHQDWLNGKEYKCKVTNKALPAPIEKTISKAKGQPREPQVYTLPPSRDELTKNQVSLTCLVKGFYPSDIAVEWESNGQPENNYKTTPPVLDSDGSFFLYSKLTVDKSRWQQGNVFSCSVMHEALHNHYTQKSLSLSPGKERKCCVECPPCP

SEQ ID NO: 74 - protein, 264 aa, Homo sapiens
METDTLLLWVLLLWVPGSTGEPKSCDKTHTCPPCPAPELLGGPSVFLFPPKPKDTLMISRTPEVTCVVVDVEFEDPEVKFNWYVDGVEVHNAKTKPREEQYNSAYRVVSVLTVLHQDWLNGKEYKCKVTNKALPAPIEKTISKAKGQPREPQVYTLPPSRDELTKNQVSLTCLVKGFYPSDIAVEWESNGQPENNYKTTPPVLDSDGSFFLYSKLTVDKSRWQQGNVFSCSVMHEALHNHYTQKSLSLSPGKERKCCVECPPCP

SEQ ID NO: 75 - protein, 264 aa, Homo sapiens
METDTLLLWVLLLWVPGSTGEPKSCDKTHTCPPCPAPELLGGPSVFLFPPKPKDTLMISRTPEVTCVVVDVQFEDPEVKFNWYVDGVEVHNAKTKPREEQYNSAYRVVSVLTVLHQDWLNGKEYKCKVTNKALPAPIEKTISKAKGQPREPQVYTLPPSRDELTKNQVSLTCLVKGFYPSDIAVEWESNGQPENNYKTTPPVLDSDGSFFLYSKLTVDKSRWQQGNVFSCSVMHEALHNHYTQKSLSLSPGKERKCCVECPPCP

SEQ ID NO: 76 - protein, 264 aa, Homo sapiens
METDTLLLWVLLLWVPGSTGEPKSCDKTHTCPPCPAPELLGGPSVFLFPPKPKDTLMISRTPEVTCVVVDVDFEDPEVKFNWYVDGVEVHNAKTKPREEQYNSAYRVVSVLTVLHQDWLNGKEYKCKVTNKALPAPIEKTISKAKGQPREPQVYTLPPSRDELTKNQVSLTCLVKGFYPSDIAVEWESNGQPENNYKTTPPVLDSDGSFFLYSKLTVDKSRWQQGNVFSCSVMHEALHNHYTQKSLSLSPGKERKCCVECPPCP

SEQ ID NO: 77 - protein, 264 aa, Homo sapiens
METDTLLLWVLLLWVPGSTGEPKSCDKTHTCPPCPAPELLGGPSVFLFPPKPKDTLMISRTPEVTCVVVDVHFEDPEVKFNWYVDGVEVHNAKTKPREEQYNSAYRVVSVLTVLHQDWLNGKEYKCKVTNKALPAPIEKTISKAKGQPREPQVYTLPPSRDELTKNQVSLTCLVKGFYPSDIAVEWESNGQPENNYKTTPPVLDSDGSFFLYSKLTVDKSRWQQGNVFSCSVMHEALHNHYTQKSLSLSPGKERKCCVECPPCP

SEQ ID NO: 78 - protein, 264 aa, Homo sapiens
METDTLLLWVLLLWVPGSTGERKCCVECPPCPEPKSCDKTHTCPPCPAPELLGGPSVFLFPPKPKDTLMISRTPEVTCVVVDVEFEDPEVKFNWYVDGVEVHNAKTKPREEQYASTYRVVSVLTVLHQDWLNGKEYKCKVTNKALPAPIEKTISKAKGQPREPQVYTLPPSREEMTKNQVSLTCLVKGFYPSDIAVEWESNGQPENNYKTTPPVLDSDGSFFLYSKLTVDKSRWQQGNVFSCSVMHEALHNHYTQKSLSLSPGK

SEQ ID NO: 79 - protein, 264 aa, Homo sapiens
METDTLLLWVLLLWVPGSTGERKCCVECPPCPEPKSCDKTHTCPPCPAPELLRGPSVFLFPPKPKDTLMISRTPEVTCVVVDVEFEDPEVKFNWYVDGVEVHNAKTKPREEQYNSTYRVVSVLTVLHQDWLNGKEYKCKVTNKALPAPIEKTISKAKGQPREPQVYTLPPSRDELTKNQVSLTCLVKGFYPSDIAVEWESNGQPENNYKTTPPVLDSDGSFFLYSKLTVDKSRWQQGNVFSCSVMHEALHNHYTQKSLSLSPGK

SEQ ID NO: 80 - protein, 263 aa, Homo sapiens
METDTLLLWVLLLVPGSTGERKCCVECPPCPEPKSCDKTHTCPPCPAPELLGGDSVFLFPPKPKDTLMISRTPEVTCVVVDVEFEDPEVKFNWYVDGVEVHNAKTKPREEQYNSTYRVVSVLTVLHQDWLNGKEYKCKVTNKALPAPIEKTISKAKGQPREPQVYTLPPSREEMTKNQVSLTCLVKGFYPSDIAVEWESNGQPENNYKTTPPVLDSDGSFFLYSKLTVDKSRWQQGNVFSCSVMHEALHNHYTQKSLSLSPGK

SEQ ID NO: 81 - protein, 264 aa, Homo sapiens; identical to SEQ ID NO: 19

SEQ ID NO: 82 - protein, 264 aa, Homo sapiens
METDTLLLWVLLLWVPGSTGEPKSCDKTHTCPPCPAPPLLRGPSVFLFPPKPKDTLMISRTPEVTCVVVAVEFEDPEVKFNWYVDGVEVHNAKTKPREEQYASTYRVVSVLTVLHQDWLNGKEYKCKVTNKALPAPIEKTISKAKGQPREPQVYTLPPSRDELTKNQVSLTCLVKGFYPSDIAVEWESNGQPENNYKTTPPVLDSDGSFFLYSKLTVDKSRWQQGNVFSCSVMHEALHNHYTQKSLSLSPGKERKCCVECPPCP

SEQ ID NO: 83 - protein, 264 aa, Homo sapiens
METDTLLLWVLLLWVPGSTGEPKSCDKTHTCPPCPAPPVAGGPSVFLFPPKPKDTLMISRTPEVTCVVVDVEFEDPEVKFNWYVDGVEVHNAKTKPREEQYASTYRVVSVLTVLHQDWLNGKEYKCKVTNKAFPAPIEKTISKAKGQPREPQVYTLPPSRDELTKNQVSLTCLVKGFYPSDIAVEWESNGQPENNYKTTPPVLDSDGSFFLYSKLTVDKSRWQQGNVFSCSVMHEALHNHYTQKSLSLSPGKERKCCVECPPCP

SEQ ID NO: 84 - protein, 264 aa, Homo sapiens
METDTLLLWVLLLWVPGSTGEPKSCDKTHTCPPCPAPELLGGDSVFLFPPKPKDTLMISRTPEVTCVVVCVEFEDPEVKFNWYVDGVEVHNAKTKPREEQYNSTYRVVSVLTVLHQDWLNGKEYKCKVTNKALPAPIEKTISKAKGQPREPQVYTLPPSRDELTKNQVSLTCLVKGFYPSDIAVEWESNGQPENNYKTTPPVLDSDGSFFLYSKLTVDKSRWQQGNVFSCSVMHEALHNHYTQKSLSLSPGKERKCCVECPPCP

SEQ ID NO: 85 - protein, 264 aa, Homo sapiens
METDTLLLWVLLLWVPGSTGEPKSCDKTHTCPPCPAPELLGGDSVFLFPPKPKDTLMISRTPEVTCVVVPVEFEDPEVKFNWYVDGVEVHNAKTKPREEQYNSTYRVVSVLTVLHQDWLNGKEYKCKVTNKALPAPIEKTISKAKGQPREPQVYTLPPSRDELTKNQVSLTCLVKGFYPSDIAVEWESNGQPENNYKTTPPVLDSDGSFFLYSKLTVDKSRWQQGNVFSCSVMHEALHNHYTQKSLSLSPGKERKCCVECPPCP

SEQ ID NO: 86 - protein, 263 aa, Homo sapiens
METDTLLLWVLLLVPGSTGERKCCVECPPCPEPKSCDKTHTCPPCPAPELLRGPSVFLFPPKPKDTLMISRTPEVTCVVVDVEFEDPEVKFNWYVDGVEVHNAKTKPREEQYNSTYRVVSVLTVLHQDWLNGKEYKCKVTNKAFPAPIEKTISKAKGQPREPQVYTLPPSREEMTKNQVSLTCLVKGFYPSDIAVEWESNGQPENNYKTTPPVLDSDGSFFLYSKLTVDKSRWQQGNVFSCSVMHEALHNHYTQKSLSLSPGK

SEQ ID NO: 87 - protein, 264 aa, Homo sapiens
METDTLLLWVLLLWVPGSTGEPKSCDKTHTCPPCPAPELLGGDSVFLFPPKPKDTLMISRTPEVTCVVVDVEFEDPEVKFNWYVDGVEVHNAKTKPREEQYNSTYRVVSVLTVLHQDWLNGKEYKCKVTNKAFPAPIEKTISKAKGQPREPQVYTLPPSRDELTKNQVSLTCLVKGFYPSDIAVEWESNGQPENNYKTTPPVLDSDGSFFLYSKLTVDKSRWQQGNVFSCSVMHEALHNHYTQKSLSLSPGKERKCCVECPPCP